European Patent Application EP 4 317 442 A1, published February 7, 2024. Title: RECOMBINANT MICROORGANISM FOR PRODUCING 2,3-BUTANEDIOL WITH REDUCED BY-PRODUCT PRODUCTION AND METHOD FOR PRODUCING 2,3-BUTANEDIOL USING THE SAME. Applicant: GS CALTEX. The sequence listing filed with the application follows.

SEQUENCE LISTING (32 sequences)

SEQ ID NO: 1 - DNA, 3001 bp, Bacillus licheniformis
atgtgggtaatgctattagcctgtgtgatcgttgttgggatcggcatttatgaaaaaaggcgccaccagcaaaatatcgatgcgctgcctgtccgagtgaacatcaacggtatacgcggaaagtccacggtgacaagattaacaacagggatattaatcgaagcaggctacaaaacagtaggaaaaacaaccgggacagacgcaaggatgatttattgggacacaccggaagagaagccgatcaaaagaaagccgcaagggccgaatatcggagagcagaaggaggttatgaaagaaacggtggaaagaggggccaatgcgattgtcagtgagtgcatggccgttaatcctgattaccaaatcatctttcaggaagaattgcttcaggctaatatcggcgtgatcgtgaacgtgctggaggatcacatggatgtgatgggaccgactttggatgaaatcgcagaagcattcacagcaaccattccttataatggacatttggttattactgatagtgagtataccgatttctttaagcaaattgcaaaagaaaggaacacaaaagtcatcgtcgcagacaattctaaaataacagatgaatacctcagacagtttgagtacatggtattccctgataatgcgtctcttgcgctcggtgtagctcaagcgttgggcattgacgaagaaaccgcctttaaaggcatgctgaatgcgccgcctgatccgggagccatgagaattctgccgctgatgaacgccaagaatcccggacatttcgtcaacggttttgcggccaatgacgcagcttccactttaaacatttggaagcgtgtaaaagaaataggctatcctacggatcagccgatcgtcattatgaactgccgcgccgacagggtagacagaacacagcagtttgcggaagatgtccttccttatattgaagcaagtgaacttgtgctgattggagaaacaacagagccgatcgtcaaagcatatgaagcaggcaaaattcctgcggacaagctgtttgattttgagcacaaatcaacggaagaaatcatgttcatgctgaaaaacaagcttgagggccgcgttatttacggagtcggaaatatccacggagcagcggagcctctcattgaaaaaatacaagattacaagattaagcagctcgttagctaggaggaagaaaacacaatgtttggatcagatttatatatcgccctcattttaggagtcttactcagtttgatttttgcggagaaaacgggaattgtaccagccggcctcgtcgtaccgggttatttgggacttgtcttcaatcagccgattttcatgctgctcgttctttttgtcagtttgctgacgtatgtcatcgtgaaattcggactttccaaaattatgattctatacggacgcagaaaattcgcagcaatgctgattacgggaattcttttgaaaatcggttttgattttatatatccggtgatgccgtttgagattgccgaattcaggggaatcggaatcatcgtgccggggctgatcgccaataccattcaaagacagggattaacgattacgcttggaagtacgcttttattgagcggagcaacattcgtcattatgtatgcttactatctaatctaaagttaggtgtgtcaaatcgatgaaaaaacaactgaactttcaggaaaaactgctgaagttgacgaagcaggagaaaaagaaaacaaacaagcacgtctttatcgtattgcccgttattttctgtttaatgtttgtctttacttgggtcggaagcgccaaaactccttcgcaaatggacaaaaaagaagatgccaagcttacagctacttttgttggcgatatcatgatgggaagaaacgtagaaaaagtgacaaacttgcacggttcggaaagtgtcttcaaaaatgtgaagccgtactttaatgtgtcagattttatcacaggaaactttgaaaaccctgtaaccaatgcaaaggactatcaagaggcagaaaagaacatccatctgcaaacgaatcaagaatcagtcgaaacattgaaaaagctgaacttcagcgtactgaattttgccaacaaccatgcgatggactacggggaagacggtttgaaggatacgctcaataaattttcaaatgagaatctggagcttgtcggagcaggaaataatcttgaagacgcgaaacagcacgtatcctatcagaatgtgaacggcgtaaaaattgcaacgctcggttttacagacgtctacacaaagaactttacagccaaaaagaacagaggcggagtgctgccgctcagtccgaaaatctttattccaatgattgcggaagcatcgaaaaaagcggatcttgtccttgtccatgtgcactggggacaagaatatgacaatgaaccgaacgacagacagaaggatctggccaaggcgattgcagatgccggagcagatgtcatcatcggcgctcatccccatgttctcgaaccgatcgaagtgtataacggtactgtgattttctacagcctcggcaactttgtatttgatcagggctggtcaagaacacgggacagcgcgcttgtacaataccatttaatgaatgacggcaaagggcgttttgaggtaacgcctctcaacattcgcgaagcaacgccgacgcctttaggcaagagcgacttcttaaaacgaaaagcgatcttccgtcaattgacaaaaggaacaaacctcgactggaaagaagagaacggaaaattaacgtttgaagtcgatcatgcggacaagctgaaaaaataataaaaacggagtggtgaacaaatgaaatttgtcagagccatttggccgttcgtaggtttagttttgatcattgcattcatgtctgctttcaagtattctgatgaattgtcaaacgatgaaaaagctaaaatctctacggagatccaaaaagtgaatcagcaggatcaaacaacagaaaacaagcaataa

SEQ ID NO: 2 - DNA, 792 bp, Bacillus licheniformis
aagccttctcctctctatttgtgtaaccgtttacataaagattatcacgatccatttaaaatcacaataaaaaaatggatgaacactgaaattttagaccgggctgggatatcgagacatatataggggcgtttaatggcgaatacagtaacaatgagaatagtaagaaaaattaaaaatgttaaagtttgatgaattatcattgaaaaaaattaatggctttttaaatcctaggattttaacctaaaatctgaagaaataaggtggatcgaacgactcacaaaatatttggatttgtcaatgaatcccgctttatgctaaaagagattttcattttttgatagatggtctgattgtcataggacggatttgttttgaagagggaacattggtgactttttaacctgttcgaaaagagcgaaaatactaaaagaaaagagagatcccggctgacagcccatttaaaggggattgcggacgggggaaaaaagagatcctgaatccatccttcaacctttcatctgaaatagggagaaaagtacaaaaatcataatgtcgaattttgaaagcgcatacttaaaacgctgacaaaaatctgataggaattaagaactttcgatttccaaaaatatcaataaaaagataggcattaatgactcgggcgaggtgatctttgtcacggaaaatttcgtcgtcttctgttacataatgccgattgtgatttcatagtgaacctatatactgatgaatgaatttacatatcagattccaagaaggagatgtagacaaaca

SEQ ID NO: 3 - DNA, 46 bp, Artificial Sequence
  nucleotide sequence of primer for amplifying homologous region 1 of pgsBCAE
agacagggccaacgaggccaagccttctcctctctatttgtgtaac

SEQ ID NO: 4 - DNA, 40 bp, Artificial Sequence
  nucleotide sequence of primer for amplifying homologous region 1 of pgsBCAE
cggcactctcttttgcactgtgtttgtctacatctccttc

SEQ ID NO: 5 - DNA, 735 bp, Bacillus licheniformis
cagtgcaaaagagagtgccgccggcgctctcttttttgtgtgctgatcccggttataaaagacctgtgaaaagcgaccggtttgaaagggaaacacgacaattttcttaaccggtcagtgtataaagttttatagaaaatcaggaggatatatacatggttttggggttcatgtttattgtattcttttgaagggaataaaaactgacaaatttcgactgaagcaaaatttgaaaatgcatcaccttaccaattcgggatgggaaccgcacctcatgttcatgacctctttagaatatttcccttcatctttttaatctgcgcttaggtgaaaaagctgatcatgctgtgctgagcgtttcttctcgctatgacgctgctgtacatgcaaaaaaagtcctttaaatatcccagttgaatgacgatgaaagaggaaagaagaggaggaacagatcaattgataaaaaaagcggcaaacaaaaagttggttttgttttgtggaattgcggtgctttggatgtctttatttttaacgaatcataatgatgtacgcgccgatacgatcggcgagaaaatagcggaaactgccagacagcttgagggtgcgaaatacagctacggcggagagaagccgaaaacggggtttgactcgtcaggctttgtgcaatatgtgtttcaatcgctcgatattacgcttccgagaacggtaaaggaacaatcgactcttgggagcagt

SEQ ID NO: 6 - DNA, 40 bp, Artificial Sequence
  nucleotide sequence of primer for amplifying homologous region 2 of pgsBCAE
gaaggagatgtagacaaacacagtgcaaaagagagtgccg

SEQ ID NO: 7 - DNA, 43 bp, Artificial Sequence
  nucleotide sequence of primer for amplifying homologous region 2 of pgsBCAE
agacagggccttattggccactgctcccaagagtcgattgttc

SEQ ID NO: 8 - DNA, 1527 bp, Artificial Sequence
  nucleotide sequence of DNA fragment comprising homologous region 1 and 2 of pgsBCAE
aagccttctcctctctatttgtgtaaccgtttacataaagattatcacgatccatttaaaatcacaataaaaaaatggatgaacactgaaattttagaccgggctgggatatcgagacatatataggggcgtttaatggcgaatacagtaacaatgagaatagtaagaaaaattaaaaatgttaaagtttgatgaattatcattgaaaaaaattaatggctttttaaatcctaggattttaacctaaaatctgaagaaataaggtggatcgaacgactcacaaaatatttggatttgtcaatgaatcccgctttatgctaaaagagattttcattttttgatagatggtctgattgtcataggacggatttgttttgaagagggaacattggtgactttttaacctgttcgaaaagagcgaaaatactaaaagaaaagagagatcccggctgacagcccatttaaaggggattgcggacgggggaaaaaagagatcctgaatccatccttcaacctttcatctgaaatagggagaaaagtacaaaaatcataatgtcgaattttgaaagcgcatacttaaaacgctgacaaaaatctgataggaattaagaactttcgatttccaaaaatatcaataaaaagataggcattaatgactcgggcgaggtgatctttgtcacggaaaatttcgtcgtcttctgttacataatgccgattgtgatttcatagtgaacctatatactgatgaatgaatttacatatcagattccaagaaggagatgtagacaaacacagtgcaaaagagagtgccgccggcgctctcttttttgtgtgctgatcccggttataaaagacctgtgaaaagcgaccggtttgaaagggaaacacgacaattttcttaaccggtcagtgtataaagttttatagaaaatcaggaggatatatacatggttttggggttcatgtttattgtattcttttgaagggaataaaaactgacaaatttcgactgaagcaaaatttgaaaatgcatcaccttaccaattcgggatgggaaccgcacctcatgttcatgacctctttagaatatttcccttcatctttttaatctgcgcttaggtgaaaaagctgatcatgctgtgctgagcgtttcttctcgctatgacgctgctgtacatgcaaaaaaagtcctttaaatatcccagttgaatgacgatgaaagaggaaagaagaggaggaacagatcaattgataaaaaaagcggcaaacaaaaagttggttttgttttgtggaattgcggtgctttggatgtctttatttttaacgaatcataatgatgtacgcgccgatacgatcggcgagaaaatagcggaaactgccagacagcttgagggtgcgaaatacagctacggcggagagaagccgaaaacggggtttgactcgtcaggctttgtgcaatatgtgtttcaatcgctcgatattacgcttccgagaacggtaaaggaacaatcgactcttgggagcagt

SEQ ID NO: 9 - DNA, 1449 bp, Bacillus licheniformis
atgaacatcaaaaacattgctaaaaaagcgtcagccttaaccgttgctgcggcactgctggccggaggtgcgccgcaaacctttgcaaaagaaacgcaggattacaagaaaagctacggattttctcatatcacaagacatgacatgctgaaaattcccgagcagcaaaagagcgaacaatttaaagttcctcaattcgatccgaaaacaatcaaaaacatcccttctgcaaaagggtataacaaaaatggagagctgatcgatttagacgtatgggacagctggccgctgcaaaatgccgacgggacggttgctacataccacggctacaatcttgttttcgcgctggcgggcgatccgaaagacgtcgatgacacatccatctatttgttctatcaaaagaaaggcgaaacttctatcgacagctggaaaaacgccggcagagtgtttaaagacagcgacaaatttgttccagacgatccgtacctcaaacatcaaacacaggaatggtcaggttctgccacgctgacaaaagacggaaaagtccgactgttttacacagctttttccggcacgcaatacggcaagcagacgctgacaacagctcaggtcaatttctctcagccggattcggacacgctcaaaattgacggtgtagaagatcataaatcggtctttgacggcgccgacggcacggtataccaaaacgttcagcaattcattgacgaaggaaactacagctccggcgacaaccatacgatgagagacccgcattatgtggaagaccgcggccataaatatctcgtatttgaagccaatacgggaacaaaaaccggctaccaaggagaagactccctattcaacagagcctactacgggggcagcaagaagttctttaaagaagaaagcagcaagctgctgcaaggtgcgaacaaaaagaacgcttcgctggctaacggcgctctcggaatcatcgaattaaataacgattatacactgaaaaaagtcatgaagcctttgatcgcctccaatacggtgacagatgaaatcgaacgggccaacctcttcaaaatgaatggaaaatggtatctgttcacagattcaagaggatcaaaaatgacaattgacggcatcggttcaaaagacatttatatgctcggctatgtatcaggttcattaaccggaccattcaagcctttaaacaaatccggacttgttttgcatatggaccaggattacaatgacatcacgtttacttattcacactttgccgtaccgcagaaaaaaggcgacgaagtcgtcattacaagctacatcacaaacagagggatttcgaacgagcatcacgccacgtttgcaccaagctttttgctgaagatcaaaggatcaaaaacatccgttgtcaaaaacagcatccttgaacagggacaactaacggtaaacaaataa

SEQ ID NO: 10 - DNA, 697 bp, Bacillus licheniformis
gattacctgcacgtatcactggttgatttccggtccttgccgcgcaggggtgcagacagatcccgcgcaaggatggaactgatcaaagaagccgtccaagaccgtctcccactgatcggagccgggcaagtacacacaccggaagacgcccttcaagcgctggaaacaggagccgatctcatcggaatcgggcggggtctcctgatggatccggagtggctacaaaaagttcgagccggaaaagaggacgatattcaaacaaccctgtcaagacatgatcagcggaagctcgcaattccagatgccttttgggaaagtataccgatgtatattgatttcagcgattgacgattcccgcttatacagactatagattcatataaaaaaggtgtctttccgcttaaaatcggtgtcatttgcataaaaatgtataggaaaagaggaacttagaccagttgagtcccagagatgagtatattagaatgatggtaattcaatatcgtcgggattgttactgtctaagcaggcaagacctaaaatgtgtgaagggcgaaatctatcttttgcctatatgaacttgcacattttaggtcttttttctgttcttcaggacaatgccgcagttaggagggatgattgggaacgttcatgttgtcagaagcaatctattacatattgaaaaagggaggaaatattg

SEQ ID NO: 11 - DNA, 46 bp, Artificial Sequence
  nucleotide sequence of primer for amplifying homologous region 1 of sacB
agacagggccaacgaggccgctagcgattacctgcacgtatcactg

SEQ ID NO: 12 - DNA, 41 bp, Artificial Sequence
  nucleotide sequence of primer for amplifying homologous region 1 of sacB
tttccttcgttcgttcaatatttcctccctttttcaatatg

SEQ ID NO: 13 - DNA, 644 bp, Bacillus licheniformis
aacgaacgaaggaaaatgccggtgaacatcggcattttctttcgtatgtcatcttagaataaagcggggaattttcttgaagaaggcagtatataagcggatcagcattttaactgtttgtcttggaatcttcatcatgatatttctttcagtccgggaaacagaaaaaaagggagaatctccggatacaccggaatatcgtgcagctttccatttgacaacccctgacaaatggaaaaacgaccctcaaaaacccgtctatttcaatggagaatatcattactactacctctataaccgagactatccggacggcaatggaacagagtggcgccacgcagtatcagatgatctcgtccactggcaggataaaggggttgccattccgaaatatacgaataaaaatggcgatccctggtccggttctgtcgttgtcgactcaaaaaacacagccggcttcggcaaagggacgatcgtggcggttatgacgcagccgtcggccaatgacgggaaggaagagcaatttttatggtacagccaaaatggaggaaaaacatttaaaccttacggtgaagagccggtcttgcctaatccgggcaccgtcgatttcagagatccgaaagtgatctgggatgaacaggatg

SEQ ID NO: 14 - DNA, 35 bp, Artificial Sequence
  nucleotide sequence of primer for amplifying homologous region 2 of sacB
agggaggaaatattgaacgaacgaaggaaaatgcc

SEQ ID NO: 15 - DNA, 45 bp, Artificial Sequence
  nucleotide sequence of primer for amplifying homologous region 2 of sacB
agacagggccttattggcccttaagcatcctgttcatcccagatc

SEQ ID NO: 16 - DNA, 1341 bp, Artificial Sequence
  nucleotide sequence of DNA fragment comprising homologous region 1 and 2 of sacB
gattacctgcacgtatcactggttgatttccggtccttgccgcgcaggggtgcagacagatcccgcgcaaggatggaactgatcaaagaagccgtccaagaccgtctcccactgatcggagccgggcaagtacacacaccggaagacgcccttcaagcgctggaaacaggagccgatctcatcggaatcgggcggggtctcctgatggatccggagtggctacaaaaagttcgagccggaaaagaggacgatattcaaacaaccctgtcaagacatgatcagcggaagctcgcaattccagatgccttttgggaaagtataccgatgtatattgatttcagcgattgacgattcccgcttatacagactatagattcatataaaaaaggtgtctttccgcttaaaatcggtgtcatttgcataaaaatgtataggaaaagaggaacttagaccagttgagtcccagagatgagtatattagaatgatggtaattcaatatcgtcgggattgttactgtctaagcaggcaagacctaaaatgtgtgaagggcgaaatctatcttttgcctatatgaacttgcacattttaggtcttttttctgttcttcaggacaatgccgcagttaggagggatgattgggaacgttcatgttgtcagaagcaatctattacatattgaaaaagggaggaaatattgaacgaacgaaggaaaatgccggtgaacatcggcattttctttcgtatgtcatcttagaataaagcggggaattttcttgaagaaggcagtatataagcggatcagcattttaactgtttgtcttggaatcttcatcatgatatttctttcagtccgggaaacagaaaaaaagggagaatctccggatacaccggaatatcgtgcagctttccatttgacaacccctgacaaatggaaaaacgaccctcaaaaacccgtctatttcaatggagaatatcattactactacctctataaccgagactatccggacggcaatggaacagagtggcgccacgcagtatcagatgatctcgtccactggcaggataaaggggttgccattccgaaatatacgaataaaaatggcgatccctggtccggttctgtcgttgtcgactcaaaaaacacagccggcttcggcaaagggacgatcgtggcggttatgacgcagccgtcggccaatgacgggaaggaagagcaatttttatggtacagccaaaatggaggaaaaacatttaaaccttacggtgaagagccggtcttgcctaatccgggcaccgtcgatttcagagatccgaaagtgatctgggatgaacaggatg

SEQ ID NO: 17 - DNA, 960 bp, Bacillus licheniformis
atgagaaaccaaaaagtcaatcgtacagttttgatcggtgcgggttttgttggaagcagctatgcatttacgttaattaaccaaggtatcacagacgaacttgtgatcattgatttaaataaagacaaagcaatgggcgatgttatggatctcaaccacggtaaagcatttgctccgcatcctgtgaaaacatggtacggcacatatgatgactgcaaagaagctgatattgtctgcgtatgcgccggagcgaaccaaaagccgggtgaaacccgccttgatctagtcgaaaagaacttgaaaatttttaaaggaatcatcggagaagtcatggccagcggttttgacggcatcttcctcgtcgctacaaaccctgtcgacatcttgacttatgcgacttggaaattcagcggccttccgaaagaacgcgtcatcggaagcggcacaacgcttgacactgcccgtttccgctacttgctcagcgagtatttcggtgtcgctgcccacaatgcgcacggctatatcattggtgaacacggagatacggagctgcctgtctggagccatgcgaatatcggcggagttcccgtcagcgacttgctgaaaagaaatgagaaatacaaagcggaagatctagatgaactgtttgacaatgtaaaaaacgccgcttaccacattattgagaaaaaaggcgcgacatactacggagttgccatgagcctcgcacgtattacgaaagcgatttatcgaaatgaagaagcaattttgaccgtgagcgctcatcttgatggtgaatttggagaaaatgatgtttatatcggagttccggcggttgtcggccgatgcggagcgagggaaattgttgagctcgatctgaacgaaaaggaaaaacaacaattcaagcatagcgcaggtgtgttaaaagcaattctaaaaccgcattttgaactgcaggcgtaa

SEQ ID NO: 18 - DNA, 730 bp, Bacillus licheniformis
cataacaacggaatcatcgtcaccagcattccgccaacagccgtctttttcggtccgaaacggtcggttaaaatgccgagcgcaatccggaaaaacgatccggccaaagtaggtatggcgacaatcaatccgacctgtgaaggcgataaatcaaaatcagccgtaacataaacaccaagcgcccccagcaacacccaaatcataaagctgacatcgaaatataaaaaagatgacaacaaggaaggcgcgtgtccgctcttcctcaaatccgccaatttcaattgcaacactccccatccgatagattctagaatttatcatgacaaaatcgaatagggttggcagtatttttgtaagctttactaacaaactaaaagattgaatatttaaaatgttagtttggacagcactatagcaggcgataattgaattatgctgaagaatagtggtgttatgagcgctgaaaatgggaaaccttatattgatataggcccgatgcacttgcagataaaaccgtcttttgcaacgcgtttatcaatttttctttagacataaggcatatttttaccagaaaatgtacaaatttaaggaagaaatacgtggagacacaaaatagacataaataaaaatgtatatcacttgaaaaagtatgtgaagtattgcacaatatgaatgtgaagaatttcacaaacagcttagtttaaaacaaacggcaaaggaatgatgagtc

SEQ ID NO: 19 - DNA, 43 bp, Artificial Sequence
  nucleotide sequence of primer for amplifying homologous region 1 of ldh
agacagggccaacgaggcccataacaacggaatcatcgtcacc

SEQ ID NO: 20 - DNA, 39 bp, Artificial Sequence
  nucleotide sequence of primer for amplifying homologous region 1 of ldh
cttcatggtgttcaggactcatcattcctttgccgtttg

SEQ ID NO: 21 - DNA, 699 bp, Bacillus licheniformis
ctgaacaccatgaagatactaacatcatgaagattgcgagatgatgaaaatgtggcagcagatatacgatccgtttggaaatctgtttatcagcgcttttgccgccatactgccgattcttttctttcttcttgcactgaccgtgttgaagatgaaaggaatcattgcgtcatttttgacgctggcggtcagctttattgtagcggtgttcttctttcacatgccggctgcgaaagctgtctccgccgttttacttggaattgctaacggcctttggccgatcggatatattgtcctgatggctgtatggctttacaaaatttctgtcaaaaccggaaagtttaaagtgatcagagcgagcattgccggaatttcgtccgaccagcggcttcagctattgctgatcgggttcagttttaacgcctttttggaaggtgcggcaggcttcggtgtgccgattgcgatcagcgccgttcttcttgtcgagcttggttttaaacctttgaaagcggcatccctatgtttaatagcgaatgcggcatccggagcctttggagccatcggaattccggttatcacaggagcgcagatgggaggcttaacaccggttgagctttccagaacgctcgctttgatgctgccggtcatcgctttctttgtcccgttcctgctcgttttcatattggacgggtttaaagg

SEQ ID NO: 22 - DNA, 44 bp, Artificial Sequence
  nucleotide sequence of primer for amplifying homologous region 2 of ldh
aaggaatgatgagtcctgaacaccatgaagatactaacatcatg

SEQ ID NO: 23 - DNA, 45 bp, Artificial Sequence
  nucleotide sequence of primer for amplifying homologous region 2 of ldh
agacagggccttattggcccctttaaacccgtccaatatgaaaac

SEQ ID NO: 24 - DNA, 1429 bp, Artificial Sequence
  nucleotide sequence of DNA fragment comprising homologous region 1and 2 of ldh
cataacaacggaatcatcgtcaccagcattccgccaacagccgtctttttcggtccgaaacggtcggttaaaatgccgagcgcaatccggaaaaacgatccggccaaagtaggtatggcgacaatcaatccgacctgtgaaggcgataaatcaaaatcagccgtaacataaacaccaagcgcccccagcaacacccaaatcataaagctgacatcgaaatataaaaaagatgacaacaaggaaggcgcgtgtccgctcttcctcaaatccgccaatttcaattgcaacactccccatccgatagattctagaatttatcatgacaaaatcgaatagggttggcagtatttttgtaagctttactaacaaactaaaagattgaatatttaaaatgttagtttggacagcactatagcaggcgataattgaattatgctgaagaatagtggtgttatgagcgctgaaaatgggaaaccttatattgatataggcccgatgcacttgcagataaaaccgtcttttgcaacgcgtttatcaatttttctttagacataaggcatatttttaccagaaaatgtacaaatttaaggaagaaatacgtggagacacaaaatagacataaataaaaatgtatatcacttgaaaaagtatgtgaagtattgcacaatatgaatgtgaagaatttcacaaacagcttagtttaaaacaaacggcaaaggaatgatgagtcctgaacaccatgaagatactaacatcatgaagattgcgagatgatgaaaatgtggcagcagatatacgatccgtttggaaatctgtttatcagcgcttttgccgccatactgccgattcttttctttcttcttgcactgaccgtgttgaagatgaaaggaatcattgcgtcatttttgacgctggcggtcagctttattgtagcggtgttcttctttcacatgccggctgcgaaagctgtctccgccgttttacttggaattgctaacggcctttggccgatcggatatattgtcctgatggctgtatggctttacaaaatttctgtcaaaaccggaaagtttaaagtgatcagagcgagcattgccggaatttcgtccgaccagcggcttcagctattgctgatcgggttcagttttaacgcctttttggaaggtgcggcaggcttcggtgtgccgattgcgatcagcgccgttcttcttgtcgagcttggttttaaacctttgaaagcggcatccctatgtttaatagcgaatgcggcatccggagcctttggagccatcggaattccggttatcacaggagcgcagatgggaggcttaacaccggttgagctttccagaacgctcgctttgatgctgccggtcatcgctttctttgtcccgttcctgctcgttttcatattggacgggtttaaagg

SEQ ID NO: 25 - DNA, 651 bp, Bacillus licheniformis
atgaagaaatgggcatttgtatcagactttgatgggacgatttccaaacaggatttttactggatggtcattgataaatattttcccgaaggccgtgaattgttcaagaagtggaagtccggagaattaaaagatatcgaatttttgggaaccgtttttgcttcgattaatcaaagcgaacaaaaaatcattgatgacatccattccataccgattgatgaatatgtgcctgacttcattcagcatgtccagaaaagcggcggcgacttctacattttaagcgccggcacggattattacattcattatattttaaagaaatacgggattacagacgttgaggtctattcaaataaaggcttttttaaagaagacaatgttcatatggacattgatgagaatcattggcattactctgagcgctatgggattgataaatcaaaggtcattcaaaagctgaaagaagagtatgagacggtttattttgcaggcgacagtgaaccggattcgcacccggctaaatttgcggatgttacgtttgcaaaggatgcgctccaggatttgctgcgtcagcagggggtgccatttgtagccgttgaaacatttgaagacattgaacaatatcttaaagaaaaagggcggatcgtctaa

SEQ ID NO: 26 - DNA, 746 bp, Bacillus licheniformis
cctaagtgataatgattcgcattatcaatgtaaatatagcagatcaatccctctctcgtctatcactttttttgctaagtatgattagtgtggttttggttaatttgttactataaacagaaaaaggactgatgagagatggcagaaacgaacccggtgatcaaaaaattgcagttcaaggataatggacagcctgtactgattgtgaatccgcctgaggcatacagcggcgtcatcgctgaatttcaaggccctgttcatcatcacgccgaatcggaccaatatgattttgttcaggtattcgcagcgaccaacgcaaagctgcaggctttagccaaggaggctgaacgtcatttggcggaagacggtctgttttggctttgctacccgaaaaaatcatcgaaagtctacaaaggatcggactgcagccgcgatacagtagccggactgcttgcagaccagggctatgaaccggttcgccaaattgcaattgatgaagactggtctgcgctcagatttcgcaaggcggaaaacatcaaaacgatgaagcggaaatttgccgtaacagagaaaggtaagcagcgtacagatcaagaatgattatatacgcctcctttcagggggacgaatattcagcttgtgaacgaaagtacacaaaaaagaaataatattatgttcaatgattcacaaactttttgtataatgaatctaatcttttaaaataccatagaaaagaggtatgcagc

SEQ ID NO: 27 - DNA, 45 bp, Artificial Sequence
  nucleotide sequence of primer for amplifying homologous region 1 of dgp
agacagggccaacgaggcccctaagtgataagtattcgcattatc

SEQ ID NO: 28 - DNA, 37 bp, Artificial Sequence
  nucleotide sequence of primer for amplifying homologous region 1 of dgp
cggcattagacgatcgctgcatacctcttttctatgg

SEQ ID NO: 29 - DNA, 723 bp, Bacillus licheniformis
gatcgtctaatgccgcgccaggttaccagcatagccatccccgcggttttggacattagtgagggcgtgcttggccggttggatgagatattgagaaaacatcagtttgacaaggcgatcatgttttttgacgatttttcctatcagcagtatgagcattcactgaaaaccgcatttcaacatgttaaagttgaagccgttctgctgccgtccaatctggacatacaggagcttttgaagcgggcattttcgatcgggaattgcgatgtcattattgccatgggcggcgggtatgttgtggactgcggaaaatacatcgccttttccaagcggaccccgttcatcagcattccgacgtcggcatccaatgacgggtttgcgagcagcaattgctcgcttcaggtcgaaggaaaaaaaacaaccgttccggcaagggttccctacggaatcatagctgatttgagcattattcaaaaagcgccggattgctttattttggcggggatcggagatttgatgtccaatattacggccctttatgattgggagtttgaggagcggcacggggtcggcgatgtaaatgcgtttgcgtcgatgctcagcaagaaagcggtcaacagctttgtccgtacgccgatgcaggatattaaacagccgatcttcttaaaagagcttgtcagttctttgacaatgggcggcatcgctacggaaatcagcggaaac

SEQ ID NO: 30 - DNA, 33 bp, Artificial Sequence
  nucleotide sequence of primer for amplifying homologous region 2 of dgp
aaagaggtatgcagcgatcgtctaatgccgcgc

SEQ ID NO: 31 - DNA, 46 bp, Artificial Sequence
  nucleotide sequence of primer for amplifying homologous region 2 of dgp
agacagggccttattggccgtcaaagaactgacaagctcttttaag

SEQ ID NO: 32 - DNA, 1469 bp, Artificial Sequence
  nucleotide sequence of DNA fragment comprising homologous region 1 and 2 of dgp
cctaagtgataatgattcgcattatcaatgtaaatatagcagatcaatccctctctcgtctatcactttttttgctaagtatgattagtgtggttttggttaatttgttactataaacagaaaaaggactgatgagagatggcagaaacgaacccggtgatcaaaaaattgcagttcaaggataatggacagcctgtactgattgtgaatccgcctgaggcatacagcggcgtcatcgctgaatttcaaggccctgttcatcatcacgccgaatcggaccaatatgattttgttcaggtattcgcagcgaccaacgcaaagctgcaggctttagccaaggaggctgaacgtcatttggcggaagacggtctgttttggctttgctacccgaaaaaatcatcgaaagtctacaaaggatcggactgcagccgcgatacagtagccggactgcttgcagaccagggctatgaaccggttcgccaaattgcaattgatgaagactggtctgcgctcagatttcgcaaggcggaaaacatcaaaacgatgaagcggaaatttgccgtaacagagaaaggtaagcagcgtacagatcaagaatgattatatacgcctcctttcagggggacgaatattcagcttgtgaacgaaagtacacaaaaaagaaataatattatgttcaatgattcacaaactttttgtataatgaatctaatcttttaaaataccatagaaaagaggtatgcagcgatcgtctaatgccgcgccaggttaccagcatagccatccccgcggttttggacattagtgagggcgtgcttggccggttggatgagatattgagaaaacatcagtttgacaaggcgatcatgttttttgacgatttttcctatcagcagtatgagcattcactgaaaaccgcatttcaacatgttaaagttgaagccgttctgctgccgtccaatctggacatacaggagcttttgaagcgggcattttcgatcgggaattgcgatgtcattattgccatgggcggcgggtatgttgtggactgcggaaaatacatcgccttttccaagcggaccccgttcatcagcattccgacgtcggcatccaatgacgggtttgcgagcagcaattgctcgcttcaggtcgaaggaaaaaaaacaaccgttccggcaagggttccctacggaatcatagctgatttgagcattattcaaaaagcgccggattgctttattttggcggggatcggagatttgatgtccaatattacggccctttatgattgggagtttgaggagcggcacggggtcggcgatgtaaatgcgtttgcgtcgatgctcagcaagaaagcggtcaacagctttgtccgtacgccgatgcaggatattaaacagccgatcttcttaaaagagcttgtcagttctttgacaatgggcggcatcgctacggaaatcagcggaaac